European Patent Application EP 4 541 909 A1, published April 23, 2025. Title: Diagnostic Biomarker For Prognosis and Target for Therapy of Diffuse Type Gastric Cancer. Applicant: Korea Research Institute of Bioscience and Biotechnology INDUSTRY-ACADEMIC COOPERATION FOUNDATION YONSEI UNIVERSITY. The sequence listing filed with the application follows.

SEQUENCE LISTING (4 sequences)

SEQ ID NO: 1 - RNA, 21 nt, Artificial Sequence
  siSYT11
gcagaaagcgcauugccaatt

SEQ ID NO: 2 - RNA, 21 nt, Artificial Sequence
  siScramble
ccuacgccaccaauuucgutt

SEQ ID NO: 3 - RNA, 19 nt, Artificial Sequence
  SYT11-ASO
uuggcaatgcgctttctgc

SEQ ID NO: 4 - RNA, 19 nt, Artificial Sequence
  NC-ASO
cctacgccaccaatttcgu